European Patent Application EP 4 386 002 A1, published June 19, 2024. Title: IL-11 HUMANIZED ANTIBODY AND APPLICATION THEREOF. Applicant: Sunshine Lake Pharma Co., Ltd. Application EP. The sequence listing filed with the application follows.

SEQUENCE LISTING (123 sequences)

SEQ ID NO: 1-3 - skipped (3 entries)

SEQ ID NO: 4 - protein, 8 aa, synthetic construct
DYTFTNYW

SEQ ID NO: 5 - protein, 8 aa, synthetic construct
IYPGGGYT

SEQ ID NO: 6 - protein, 12 aa, synthetic construct
ARVRSGNDALDF

SEQ ID NO: 7-36 - skipped (30 entries)

SEQ ID NO: 37 - protein, 10 aa, synthetic construct
ESVDEYGISF

SEQ ID NO: 38 - skipped

SEQ ID NO: 39 - protein, 9 aa, synthetic construct
QQSKEVPWT

SEQ ID NO: 40-66 - skipped (27 entries)

SEQ ID NO: 67 - protein, 25 aa, synthetic construct [sequence omitted]

SEQ ID NO: 68 - protein, 17 aa, synthetic construct
  VARIANT 10: note = X=Q or H
  VARIANT 15: note = X=M or I
LGWVRQAPGXGLEWXGH

SEQ ID NO: 69 - protein, 38 aa, synthetic construct
  VARIANT 10: note = X=V or A
  VARIANT 12: note = X=M or L
  VARIANT 14: note = X=R or A
  VARIANT 37: note = X=Y or F
NYNEKFKGRXTXTXDTSTSTVYMELSSLRSEDTAVYXC

SEQ ID NO: 70 - protein, 11 aa, synthetic construct
WGQGTLVTVSS

SEQ ID NO: 71 - protein, 26 aa, synthetic construct [sequence omitted]

SEQ ID NO: 72 - protein, 17 aa, synthetic construct
  VARIANT 4: note = X=Y or F
MNWXQQKPGQAPRLLIY

SEQ ID NO: 73 - protein, 36 aa, synthetic construct
  VARIANT 33: note = X=V or M
  VARIANT 35: note = X=Y or F
NQGSGIPARFSGSGSGTDFTLTISSLEPEDFAXYXC

SEQ ID NO: 74 - protein, 10 aa, synthetic construct
FGGGTKLEIK

SEQ ID NO: 75 - protein, 119 aa, synthetic construct
QVQLVQSGAEVKKPGASVKVSCKASDYTFTNYWLGWVRQAPGQGLEWMGHIYPGGGYTNYNEKFKGRVTMTRDTSTSTVYMELSSLRSEDTAVYYCARVRSGNDALDFWGQGTLVTVSS

SEQ ID NO: 76 - protein, 119 aa, synthetic construct
QVQLVQSGAEVKKPGASVKVSCKASDYTFTNYWLGWVRQAPGQGLEWIGHIYPGGGYTNYNEKFKGRVTMTADTSTSTVYMELSSLRSEDTAVYFCARVRSGNDALDFWGQGTLVTVSS

SEQ ID NO: 77 - protein, 119 aa, synthetic construct
QVQLVQSGAEVKKPGASVKVSCKASDYTFTNYWLGWVRQAPGQGLEWIGHIYPGGGYTNYNEKFKGRATLTADTSTSTVYMELSSLRSEDTAVYFCARVRSGNDALDFWGQGTLVTVSS

SEQ ID NO: 78 - protein, 119 aa, synthetic construct
QVQLVQSGAEVKKPGASVKVSCKASDYTFTNYWLGWVRQAPGHGLEWIGHIYPGGGYTNYNEKFKGRATLTADTSTSTVYMELSSLRSEDTAVYFCARVRSGNDALDFWGQGTLVTVSS

SEQ ID NO: 79 - protein, 111 aa, synthetic construct
EIVLTQSPATLSLSPGERATLSCRASESVDEYGISFMNWYQQKPGQAPRLLIYSASNQGSGIPARFSGSGSGTDFTLTISSLEPEDFAVYYCQQSKEVPWTFGGGTKLEIK

SEQ ID NO: 80 - protein, 111 aa, synthetic construct
EIVLTQSPATLSLSPGERATLSCRASESVDEYGISFMNWYQQKPGQAPRLLIYSASNQGSGIPARFSGSGSGTDFTLTISSLEPEDFAVYFCQQSKEVPWTFGGGTKLEIK

SEQ ID NO: 81 - protein, 111 aa, synthetic construct
EIVLTQSPATLSLSPGERATLSCRASESVDEYGISFMNWFQQKPGQAPRLLIYSASNQGSGIPARFSGSGSGTDFTLTISSLEPEDFAVYFCQQSKEVPWTFGGGTKLEIK

SEQ ID NO: 82 - protein, 111 aa, synthetic construct
EIVLTQSPATLSLSPGERATLSCRASESVDEYGISFMNWFQQKPGQAPRLLIYSASNQGSGIPARFSGSGSGTDFTLTISSLEPEDFAMYFCQQSKEVPWTFGGGTKLEIK

SEQ ID NO: 83 - protein, 330 aa, synthetic construct [sequence omitted]

SEQ ID NO: 84 - protein, 107 aa, synthetic construct [sequence omitted]

SEQ ID NO: 85 - protein, 449 aa, synthetic construct
QVQLVQSGAEVKKPGASVKVSCKASDYTFTNYWLGWVRQAPGQGLEWMGHIYPGGGYTNYNEKFKGRVTMTRDTSTSTVYMELSSLRSEDTAVYYCARVRSGNDALDFWGQGTLVTVSSASTKGPSVFPLAPSSKSTSGGTAALGCLVKDYFPEPVTVSWNSGALTSGVHTFPAVLQSSGLYSLSSVVTVPSSSLGTQTYICNVNHKPSNTKVDKKVEPKSCDKTHTCPPCPAPELLGGPSVFLFPPKPKDTLMISRTPEVTCVVVDVSHEDPEVKFNWYVDGVEVHNAKTKPREEQYNSTYRVVSVLTVLHQDWLNGKEYKCKVSNKALPAPIEKTISKAKGQPREPQVYTLPPSRDELTKNQVSLTCLVKGFYPSDIAVEWESNGQPENNYKTTPPVLDSDGSFFLYSKLTVDKSRWQQGNVFSCSVMHEALHNHYTQKSLSLSPGK

SEQ ID NO: 86 - protein, 449 aa, synthetic construct
QVQLVQSGAEVKKPGASVKVSCKASDYTFTNYWLGWVRQAPGQGLEWIGHIYPGGGYTNYNEKFKGRVTMTADTSTSTVYMELSSLRSEDTAVYFCARVRSGNDALDFWGQGTLVTVSSASTKGPSVFPLAPSSKSTSGGTAALGCLVKDYFPEPVTVSWNSGALTSGVHTFPAVLQSSGLYSLSSVVTVPSSSLGTQTYICNVNHKPSNTKVDKKVEPKSCDKTHTCPPCPAPELLGGPSVFLFPPKPKDTLMISRTPEVTCVVVDVSHEDPEVKFNWYVDGVEVHNAKTKPREEQYNSTYRVVSVLTVLHQDWLNGKEYKCKVSNKALPAPIEKTISKAKGQPREPQVYTLPPSRDELTKNQVSLTCLVKGFYPSDIAVEWESNGQPENNYKTTPPVLDSDGSFFLYSKLTVDKSRWQQGNVFSCSVMHEALHNHYTQKSLSLSPGK

SEQ ID NO: 87 - protein, 449 aa, synthetic construct
QVQLVQSGAEVKKPGASVKVSCKASDYTFTNYWLGWVRQAPGQGLEWIGHIYPGGGYTNYNEKFKGRATLTADTSTSTVYMELSSLRSEDTAVYFCARVRSGNDALDFWGQGTLVTVSSASTKGPSVFPLAPSSKSTSGGTAALGCLVKDYFPEPVTVSWNSGALTSGVHTFPAVLQSSGLYSLSSVVTVPSSSLGTQTYICNVNHKPSNTKVDKKVEPKSCDKTHTCPPCPAPELLGGPSVFLFPPKPKDTLMISRTPEVTCVVVDVSHEDPEVKFNWYVDGVEVHNAKTKPREEQYNSTYRVVSVLTVLHQDWLNGKEYKCKVSNKALPAPIEKTISKAKGQPREPQVYTLPPSRDELTKNQVSLTCLVKGFYPSDIAVEWESNGQPENNYKTTPPVLDSDGSFFLYSKLTVDKSRWQQGNVFSCSVMHEALHNHYTQKSLSLSPGK

SEQ ID NO: 88 - protein, 449 aa, synthetic construct
QVQLVQSGAEVKKPGASVKVSCKASDYTFTNYWLGWVRQAPGHGLEWIGHIYPGGGYTNYNEKFKGRATLTADTSTSTVYMELSSLRSEDTAVYFCARVRSGNDALDFWGQGTLVTVSSASTKGPSVFPLAPSSKSTSGGTAALGCLVKDYFPEPVTVSWNSGALTSGVHTFPAVLQSSGLYSLSSVVTVPSSSLGTQTYICNVNHKPSNTKVDKKVEPKSCDKTHTCPPCPAPELLGGPSVFLFPPKPKDTLMISRTPEVTCVVVDVSHEDPEVKFNWYVDGVEVHNAKTKPREEQYNSTYRVVSVLTVLHQDWLNGKEYKCKVSNKALPAPIEKTISKAKGQPREPQVYTLPPSRDELTKNQVSLTCLVKGFYPSDIAVEWESNGQPENNYKTTPPVLDSDGSFFLYSKLTVDKSRWQQGNVFSCSVMHEALHNHYTQKSLSLSPGK

SEQ ID NO: 89 - protein, 218 aa, synthetic construct
EIVLTQSPATLSLSPGERATLSCRASESVDEYGISFMNWYQQKPGQAPRLLIYSASNQGSGIPARFSGSGSGTDFTLTISSLEPEDFAVYYCQQSKEVPWTFGGGTKLEIKRTVAAPSVFIFPPSDEQLKSGTASVVCLLNNFYPREAKVQWKVDNALQSGNSQESVTEQDSKDSTYSLSSTLTLSKADYEKHKVYACEVTHQGLSSPVTKSFNRGEC

SEQ ID NO: 90 - protein, 218 aa, synthetic construct
EIVLTQSPATLSLSPGERATLSCRASESVDEYGISFMNWYQQKPGQAPRLLIYSASNQGSGIPARFSGSGSGTDFTLTISSLEPEDFAVYFCQQSKEVPWTFGGGTKLEIKRTVAAPSVFIFPPSDEQLKSGTASVVCLLNNFYPREAKVQWKVDNALQSGNSQESVTEQDSKDSTYSLSSTLTLSKADYEKHKVYACEVTHQGLSSPVTKSFNRGEC

SEQ ID NO: 91 - protein, 218 aa, synthetic construct
EIVLTQSPATLSLSPGERATLSCRASESVDEYGISFMNWFQQKPGQAPRLLIYSASNQGSGIPARFSGSGSGTDFTLTISSLEPEDFAVYFCQQSKEVPWTFGGGTKLEIKRTVAAPSVFIFPPSDEQLKSGTASVVCLLNNFYPREAKVQWKVDNALQSGNSQESVTEQDSKDSTYSLSSTLTLSKADYEKHKVYACEVTHQGLSSPVTKSFNRGEC

SEQ ID NO: 92 - protein, 218 aa, synthetic construct
EIVLTQSPATLSLSPGERATLSCRASESVDEYGISFMNWFQQKPGQAPRLLIYSASNQGSGIPARFSGSGSGTDFTLTISSLEPEDFAMYFCQQSKEVPWTFGGGTKLEIKRTVAAPSVFIFPPSDEQLKSGTASVVCLLNNFYPREAKVQWKVDNALQSGNSQESVTEQDSKDSTYSLSSTLTLSKADYEKHKVYACEVTHQGLSSPVTKSFNRGEC

SEQ ID NO: 93 - DNA, 1353 bp, synthetic construct
  source 1..1353: mol_type = other DNA
caagtgcagctggttcagagcggagctgaggtgaagaagcctggagctagcgtgaaggtgtcttgtaaagccagcgactacacctttaccaattactggctgggctgggtcagacaggcccctggccagggcctggaatggatgggccacatctaccccggcggaggctacacaaactacaacgagaagttcaagggcagagtgacaatgaccagagatacaagcaccagcacagtgtatatggaactgtctagcctgcggagcgaggacaccgccgtgtactactgcgccagagtgcggtccggcaacgacgccctggatttctggggccagggcaccctggtgaccgtgtccagcgccagcaccaagggcccttccgtgtttccactggccccctcctctaaatccacatctggcggcaccgccgccctgggctgtctggtgaaggactacttcccagagcctgtgacagtgtcctggaactctggcgccctgacatccggcgtgcacacatttccagccgtgctgcagagctccggcctgtacagcctgtctagcgtggtgacagtgccctcctctagcctgggcacacagacctatatctgcaacgtgaatcacaagccaagcaataccaaggtggacaagaaggtggagcccaagtcctgtgataagacacacacctgccccccttgtcctgctcccgagctgctgggcggccctagcgtgttcctgtttccacccaagcctaaggacaccctgatgatctcccggacacccgaggtgacctgcgtggtggtggacgtgtctcacgaggatcctgaggtgaagttcaactggtatgtggatggcgtggaggtgcacaatgccaagaccaagcccagagaggagcagtacaactctacatatagggtggtgagcgtgctgaccgtgctgcaccaggactggctgaacggcaaggagtataagtgcaaggtgtccaataaggccctgcccgcccccatcgagaagacaatcagcaaggccaagggccagcctcgggagccacaggtgtacaccctgcctccatccagagacgagctgacaaagaaccaggtgtctctgacatgtctggtgaagggcttctatcctagcgatatcgccgtggagtgggagtccaatggccagccagagaacaattacaagaccacaccccctgtgctggactccgatggctccttctttctgtattccaagctgaccgtggataagtctcggtggcagcagggcaacgtgttcagctgttccgtgatgcacgaagccctgcataatcactatactcagaaatccctgtccctgtcacctggaaagtgataa

SEQ ID NO: 94 - DNA, 1353 bp, synthetic construct
  source 1..1353: mol_type = other DNA
caagtgcagctggtccagagcggcgccgaggtgaaaaagcctggagctagcgtgaaggtgtcctgcaaggccagcgactacaccttcaccaactattggctgggctgggtgcggcaggcccctggacagggcctggaatggatcggccacatctaccccggaggcggctacaccaattacaacgagaagttcaagggcagagtgaccatgaccgccgatacaagcacatctacagtgtacatggaactgagcagcctgagaagcgaggatacagctgtttacttctgtgccagagtgcggtccggcaacgacgccctggacttttggggccagggcaccctggtgaccgtgtctagcgccagcaccaagggcccttccgtgtttccactggccccctcctctaaatccacatctggcggcaccgccgccctgggctgtctggtgaaggactacttcccagagcctgtgacagtgtcctggaactctggcgccctgacatccggcgtgcacacatttccagccgtgctgcagagctccggcctgtacagcctgtctagcgtggtgacagtgccctcctctagcctgggcacacagacctatatctgcaacgtgaatcacaagccaagcaataccaaggtggacaagaaggtggagcccaagtcctgtgataagacacacacctgccccccttgtcctgctcccgagctgctgggcggccctagcgtgttcctgtttccacccaagcctaaggacaccctgatgatctcccggacacccgaggtgacctgcgtggtggtggacgtgtctcacgaggatcctgaggtgaagttcaactggtatgtggatggcgtggaggtgcacaatgccaagaccaagcccagagaggagcagtacaactctacatatagggtggtgagcgtgctgaccgtgctgcaccaggactggctgaacggcaaggagtataagtgcaaggtgtccaataaggccctgcccgcccccatcgagaagacaatcagcaaggccaagggccagcctcgggagccacaggtgtacaccctgcctccatccagagacgagctgacaaagaaccaggtgtctctgacatgtctggtgaagggcttctatcctagcgatatcgccgtggagtgggagtccaatggccagccagagaacaattacaagaccacaccccctgtgctggactccgatggctccttctttctgtattccaagctgaccgtggataagtctcggtggcagcagggcaacgtgttcagctgttccgtgatgcacgaagccctgcataatcactatactcagaaatccctgtccctgtcacctggaaagtgataa

SEQ ID NO: 95 - DNA, 1353 bp, synthetic construct
  source 1..1353: mol_type = other DNA
caagtgcagctggtccagagcggcgccgaggtgaaaaagcctggcgcttctgtgaaggtgtcctgcaaggccagcgactacacatttaccaattattggctgggctgggtgcggcaggcccctggacagggcctggaatggatcggccacatctaccccggcggaggctacacaaactacaacgagaagttcaagggcagagccacactcaccgctgataccagcacaagcaccgtgtacatggaactgagcagcctgagaagcgaggacaccgccgtgtacttctgtgccagagtgcggtccggcaacgacgccctggatttctggggacagggcaccctggtgaccgtgtctagcgccagcaccaagggcccttccgtgtttccactggccccctcctctaaatccacatctggcggcaccgccgccctgggctgtctggtgaaggactacttcccagagcctgtgacagtgtcctggaactctggcgccctgacatccggcgtgcacacatttccagccgtgctgcagagctccggcctgtacagcctgtctagcgtggtgacagtgccctcctctagcctgggcacacagacctatatctgcaacgtgaatcacaagccaagcaataccaaggtggacaagaaggtggagcccaagtcctgtgataagacacacacctgccccccttgtcctgctcccgagctgctgggcggccctagcgtgttcctgtttccacccaagcctaaggacaccctgatgatctcccggacacccgaggtgacctgcgtggtggtggacgtgtctcacgaggatcctgaggtgaagttcaactggtatgtggatggcgtggaggtgcacaatgccaagaccaagcccagagaggagcagtacaactctacatatagggtggtgagcgtgctgaccgtgctgcaccaggactggctgaacggcaaggagtataagtgcaaggtgtccaataaggccctgcccgcccccatcgagaagacaatcagcaaggccaagggccagcctcgggagccacaggtgtacaccctgcctccatccagagacgagctgacaaagaaccaggtgtctctgacatgtctggtgaagggcttctatcctagcgatatcgccgtggagtgggagtccaatggccagccagagaacaattacaagaccacaccccctgtgctggactccgatggctccttctttctgtattccaagctgaccgtggataagtctcggtggcagcagggcaacgtgttcagctgttccgtgatgcacgaagccctgcataatcactatactcagaaatccctgtccctgtcacctggaaagtgataa

SEQ ID NO: 96 - DNA, 1353 bp, synthetic construct
  source 1..1353: mol_type = other DNA
caagtgcagctggttcagagcggcgccgaggtgaagaagcctggcgctagcgtgaaggtgtcttgtaaagccagcgactacacatttaccaattactggctgggatgggtccggcaggcccctggccacggcctggaatggatcggccacatctaccccggcggaggatatacaaactacaacgagaagttcaagggcagagccaccctgaccgctgatacatctacaagcaccgtgtacatggaactgagcagcctgagaagcgaggataccgccgtgtacttctgcgccagagtgcggtccggcaacgacgccctggacttctggggccagggcaccctggtgaccgtgtccagcgccagcaccaagggcccttccgtgtttccactggccccctcctctaaatccacatctggcggcaccgccgccctgggctgtctggtgaaggactacttcccagagcctgtgacagtgtcctggaactctggcgccctgacatccggcgtgcacacatttccagccgtgctgcagagctccggcctgtacagcctgtctagcgtggtgacagtgccctcctctagcctgggcacacagacctatatctgcaacgtgaatcacaagccaagcaataccaaggtggacaagaaggtggagcccaagtcctgtgataagacacacacctgccccccttgtcctgctcccgagctgctgggcggccctagcgtgttcctgtttccacccaagcctaaggacaccctgatgatctcccggacacccgaggtgacctgcgtggtggtggacgtgtctcacgaggatcctgaggtgaagttcaactggtatgtggatggcgtggaggtgcacaatgccaagaccaagcccagagaggagcagtacaactctacatatagggtggtgagcgtgctgaccgtgctgcaccaggactggctgaacggcaaggagtataagtgcaaggtgtccaataaggccctgcccgcccccatcgagaagacaatcagcaaggccaagggccagcctcgggagccacaggtgtacaccctgcctccatccagagacgagctgacaaagaaccaggtgtctctgacatgtctggtgaagggcttctatcctagcgatatcgccgtggagtgggagtccaatggccagccagagaacaattacaagaccacaccccctgtgctggactccgatggctccttctttctgtattccaagctgaccgtggataagtctcggtggcagcagggcaacgtgttcagctgttccgtgatgcacgaagccctgcataatcactatactcagaaatccctgtccctgtcacctggaaagtgataa

SEQ ID NO: 97 - DNA, 660 bp, synthetic construct
  source 1..660: mol_type = other DNA
gagatcgtgctgacacagagccctgctacactctccctgtccccaggcgagcgggccacactgtcttgtagagccagcgagagcgtcgacgagtacggcattagcttcatgaactggtatcagcagaaacctggccaggcccctagactgctgatctacagcgcctccaaccagggcagcggcatccccgctagattcagcggcagcggatctggcaccgacttcaccctgaccatcagcagcctggaacccgaggattttgccgtgtactactgccagcaatctaaggaagtgccttggaccttcggcggaggcaccaagctggaaatcaagaggacagtggccgccccaagcgtgttcatctttcccccttccgacgagcagctgaagtctggcaccgccagcgtggtgtgcctgctgaacaacttctaccctcgggaggccaaggtccagtggaaggtggataacgccctgcagtctggcaatagccaggagtccgtgaccgagcaggactctaaggatagcacatattccctgtctagcaccctgacactgagcaaggccgattacgagaagcacaaggtgtatgcctgtgaagtcacccatcaggggctgtcatcacccgtcactaagtcattcaatcgcggagaatgctgataa

SEQ ID NO: 98 - DNA, 660 bp, synthetic construct
  source 1..660: mol_type = other DNA
gagatcgtgctgacccagagccccgccaccctgtccctgagccctggcgagcgggctacactgtcttgtagagccagcgagagcgtcgacgagtacggcatctcttttatgaactggtatcagcagaaacctggacaggcccctagactgctgatctacagcgcctccaaccagggcagcggcattcctgctagattcagcggcagcggctccggcacagatttcaccctcaccatcagcagcctggaacccgaggacttcgccgtgtacttctgccagcaatctaaggaagtgccatggacattcggcggaggcaccaagctggaaatcaagaggacagtggccgccccaagcgtgttcatctttcccccttccgacgagcagctgaagtctggcaccgccagcgtggtgtgcctgctgaacaacttctaccctcgggaggccaaggtccagtggaaggtggataacgccctgcagtctggcaatagccaggagtccgtgaccgagcaggactctaaggatagcacatattccctgtctagcaccctgacactgagcaaggccgattacgagaagcacaaggtgtatgcctgtgaagtcacccatcaggggctgtcatcacccgtcactaagtcattcaatcgcggagaatgctgataa

SEQ ID NO: 99 - DNA, 660 bp, synthetic construct
  source 1..660: mol_type = other DNA
gagatcgtgctgacccagtctccagccaccctctccctgagccccggcgagcgggccacactgtcttgtagagctagcgagagcgtcgacgagtacggcatctccttcatgaactggttccagcagaaacctggccaggcccctagactgctgatctacagcgccagcaaccagggctccggaattcctgctagattcagcggctctggcagcggcacagattttaccctgacaatcagcagcctggaacccgaggactttgccgtgtacttctgccagcaaagcaaggaagtgccttggaccttcggcggaggcaccaagctggaaatcaagaggacagtggccgccccaagcgtgttcatctttcccccttccgacgagcagctgaagtctggcaccgccagcgtggtgtgcctgctgaacaacttctaccctcgggaggccaaggtccagtggaaggtggataacgccctgcagtctggcaatagccaggagtccgtgaccgagcaggactctaaggatagcacatattccctgtctagcaccctgacactgagcaaggccgattacgagaagcacaaggtgtatgcctgtgaagtcacccatcaggggctgtcatcacccgtcactaagtcattcaatcgcggagaatgctgataa

SEQ ID NO: 100 - DNA, 660 bp, synthetic construct
  source 1..660: mol_type = other DNA
gagatcgtgctgacacagagccctgctacactctccctgagccccggcgagcgggccaccctgtcttgtagagccagcgagagcgtggacgagtacggcattagcttcatgaactggtttcagcagaaacctggccaggcccctagactgctgatctacagcgcctccaaccagggctctggcatccccgctagattcagcggatctggctccggcaccgacttcaccctgaccatcagcagcctggaaccagaggattttgccatgtacttctgccagcaaagcaaggaagtgccttggaccttcggcggaggcacaaagctggaaatcaagaggacagtggccgccccaagcgtgttcatctttcccccttccgacgagcagctgaagtctggcaccgccagcgtggtgtgcctgctgaacaacttctaccctcgggaggccaaggtccagtggaaggtggataacgccctgcagtctggcaatagccaggagtccgtgaccgagcaggactctaaggatagcacatattccctgtctagcaccctgacactgagcaaggccgattacgagaagcacaaggtgtatgcctgtgaagtcacccatcaggggctgtcatcacccgtcactaagtcattcaatcgcggagaatgctgataa

SEQ ID NO: 101 - protein, 447 aa, synthetic construct
QIQLVQSGPELKKPGETVKISCKASGYTFTTNGINWVKQAAGKGLKWMGWINTNTGEPTNAEELKGRFAFSLETSASTAYLQINNLKNEDAAIYFCAREGAFGLDYWGQGTSVTVSSASTKGPSVFPLAPSSKSTSGGTAALGCLVKDYFPEPVTVSWNSGALTSGVHTFPAVLQSSGLYSLSSVVTVPSSSLGTQTYICNVNHKPSNTKVDKKVEPKSCDKTHTCPPCPAPELLGGPSVFLFPPKPKDTLMISRTPEVTCVVVDVSHEDPEVKFNWYVDGVEVHNAKTKPREEQYNSTYRVVSVLTVLHQDWLNGKEYKCKVSNKALPAPIEKTISKAKGQPREPQVYTLPPSRDELTKNQVSLTCLVKGFYPSDIAVEWESNGQPENNYKTTPPVLDSDGSFFLYSKLTVDKSRWQQGNVFSCSVMHEALHNHYTQKSLSLSPGK

SEQ ID NO: 102 - protein, 449 aa, synthetic construct
QVQLQQSGAELVRPGTSAKISCKASDYTFTNYWLGWLKQRPGHGLEWIGHIYPGGGYTNYNEKFKGKATLTADTSSSTAYMQLSSLTSEDSAVYFCARVRSGNDALDFWGQGTSVTVSSASTKGPSVFPLAPSSKSTSGGTAALGCLVKDYFPEPVTVSWNSGALTSGVHTFPAVLQSSGLYSLSSVVTVPSSSLGTQTYICNVNHKPSNTKVDKKVEPKSCDKTHTCPPCPAPELLGGPSVFLFPPKPKDTLMISRTPEVTCVVVDVSHEDPEVKFNWYVDGVEVHNAKTKPREEQYNSTYRVVSVLTVLHQDWLNGKEYKCKVSNKALPAPIEKTISKAKGQPREPQVYTLPPSRDELTKNQVSLTCLVKGFYPSDIAVEWESNGQPENNYKTTPPVLDSDGSFFLYSKLTVDKSRWQQGNVFSCSVMHEALHNHYTQKSLSLSPGK

SEQ ID NO: 103 - protein, 447 aa, synthetic construct
QIQLVQSGPELKKPGETVKISCKASGYTFTNYGMNWVKQAPGKGLKWMGWINTNTGEPTYAEEIKGRFAFSLETSASTAYLQINNLKNEDTATYFCSREGIYGMDSWGQGTSVTVSSASTKGPSVFPLAPSSKSTSGGTAALGCLVKDYFPEPVTVSWNSGALTSGVHTFPAVLQSSGLYSLSSVVTVPSSSLGTQTYICNVNHKPSNTKVDKKVEPKSCDKTHTCPPCPAPELLGGPSVFLFPPKPKDTLMISRTPEVTCVVVDVSHEDPEVKFNWYVDGVEVHNAKTKPREEQYNSTYRVVSVLTVLHQDWLNGKEYKCKVSNKALPAPIEKTISKAKGQPREPQVYTLPPSRDELTKNQVSLTCLVKGFYPSDIAVEWESNGQPENNYKTTPPVLDSDGSFFLYSKLTVDKSRWQQGNVFSCSVMHEALHNHYTQKSLSLSPGK

SEQ ID NO: 104 - protein, 451 aa, synthetic construct
QVQLKESGPGLVAPSQSLSITCTVSGFSLTSYGVHWVRQPPGKGLEWLGIIWAGGRTDYNSALVSRLNISKDNSKSQVFLKMHSLQTDDTAMYYCAREGGYDYDGDLWTTGVKEPQSPSPQASTKGPSVFPLAPSSKSTSGGTAALGCLVKDYFPEPVTVSWNSGALTSGVHTFPAVLQSSGLYSLSSVVTVPSSSLGTQTYICNVNHKPSNTKVDKKVEPKSCDKTHTCPPCPAPELLGGPSVFLFPPKPKDTLMISRTPEVTCVVVDVSHEDPEVKFNWYVDGVEVHNAKTKPREEQYNSTYRVVSVLTVLHQDWLNGKEYKCKVSNKALPAPIEKTISKAKGQPREPQVYTLPPSRDELTKNQVSLTCLVKGFYPSDIAVEWESNGQPENNYKTTPPVLDSDGSFFLYSKLTVDKSRWQQGNVFSCSVMHEALHNHYTQKSLSLSPGK

SEQ ID NO: 105 - protein, 449 aa, synthetic construct
QVQLKQSGPGLVLPSQSLSITCTVSGFSLTSYGVHWFRQSPGTGLEWLGVIWSGGITDYNATFIPRLSISKDNSKSQVFFKMNSLQADDTAIYYCARNFDGYYYSIDYWGQGTSVTVSSASTKGPSVFPLAPSSKSTSGGTAALGCLVKDYFPEPVTVSWNSGALTSGVHTFPAVLQSSGLYSLSSVVTVPSSSLGTQTYICNVNHKPSNTKVDKKVEPKSCDKTHTCPPCPAPELLGGPSVFLFPPKPKDTLMISRTPEVTCVVVDVSHEDPEVKFNWYVDGVEVHNAKTKPREEQYNSTYRVVSVLTVLHQDWLNGKEYKCKVSNKALPAPIEKTISKAKGQPREPQVYTLPPSRDELTKNQVSLTCLVKGFYPSDIAVEWESNGQPENNYKTTPPVLDSDGSFFLYSKLTVDKSRWQQGNVFSCSVMHEALHNHYTQKSLSLSPGK

SEQ ID NO: 106 - protein, 448 aa, synthetic construct
QVQLKQSGPGLVQPSQSLSITCTVSGFSLTNYGVHWVRQSPGKGLEWLGAIWRGGSTDYNAAFMSRLSITKDNSKSQVFFKMNSLQPDDTAIYYCAKNLYGPAAMDYWGQGTSVTVSSASTKGPSVFPLAPSSKSTSGGTAALGCLVKDYFPEPVTVSWNSGALTSGVHTFPAVLQSSGLYSLSSVVTVPSSSLGTQTYICNVNHKPSNTKVDKKVEPKSCDKTHTCPPCPAPELLGGPSVFLFPPKPKDTLMISRTPEVTCVVVDVSHEDPEVKFNWYVDGVEVHNAKTKPREEQYNSTYRVVSVLTVLHQDWLNGKEYKCKVSNKALPAPIEKTISKAKGQPREPQVYTLPPSRDELTKNQVSLTCLVKGFYPSDIAVEWESNGQPENNYKTTPPVLDSDGSFFLYSKLTVDKSRWQQGNVFSCSVMHEALHNHYTQKSLSLSPGK

SEQ ID NO: 107 - protein, 445 aa, synthetic construct
QIQLVQSGPELKKPGETVNISCRASGDTFTNYAVNWVKQAPGKGLKWMGWIDTYTGDPTYADDLKGRFAFSLETSATTAYLQINNLKNEDTATYFCAGDTWFAYWGQGTLVTVSAASTKGPSVFPLAPSSKSTSGGTAALGCLVKDYFPEPVTVSWNSGALTSGVHTFPAVLQSSGLYSLSSVVTVPSSSLGTQTYICNVNHKPSNTKVDKKVEPKSCDKTHTCPPCPAPELLGGPSVFLFPPKPKDTLMISRTPEVTCVVVDVSHEDPEVKFNWYVDGVEVHNAKTKPREEQYNSTYRVVSVLTVLHQDWLNGKEYKCKVSNKALPAPIEKTISKAKGQPREPQVYTLPPSRDELTKNQVSLTCLVKGFYPSDIAVEWESNGQPENNYKTTPPVLDSDGSFFLYSKLTVDKSRWQQGNVFSCSVMHEALHNHYTQKSLSLSPGK

SEQ ID NO: 108 - protein, 450 aa, synthetic construct
QVTLKESGPGILQPSQTLSLTCSFSGFSLSSSGMSVGWIRQPSGKGLEWLAHIWWSDDKSYNPALKSRLTISKDTSNNQVFLKIASVVTADTATYYCAREGSLGYGLDYWGQGTTLTVSSASTKGPSVFPLAPSSKSTSGGTAALGCLVKDYFPEPVTVSWNSGALTSGVHTFPAVLQSSGLYSLSSVVTVPSSSLGTQTYICNVNHKPSNTKVDKKVEPKSCDKTHTCPPCPAPELLGGPSVFLFPPKPKDTLMISRTPEVTCVVVDVSHEDPEVKFNWYVDGVEVHNAKTKPREEQYNSTYRVVSVLTVLHQDWLNGKEYKCKVSNKALPAPIEKTISKAKGQPREPQVYTLPPSRDELTKNQVSLTCLVKGFYPSDIAVEWESNGQPENNYKTTPPVLDSDGSFFLYSKLTVDKSRWQQGNVFSCSVMHEALHNHYTQKSLSLSPGK

SEQ ID NO: 109 - protein, 447 aa, synthetic construct
EVKLLESGGGLVQPGGSLKLSCAASGFDFRRYWMSWVRQAPGKGLEWIGQINPDSSMINYTPSLKDKFIISRDNAKNTLYLQMSEVRSEDTALYYCATYGHHATDSWGQGTSVTVSSASTKGPSVFPLAPSSKSTSGGTAALGCLVKDYFPEPVTVSWNSGALTSGVHTFPAVLQSSGLYSLSSVVTVPSSSLGTQTYICNVNHKPSNTKVDKKVEPKSCDKTHTCPPCPAPELLGGPSVFLFPPKPKDTLMISRTPEVTCVVVDVSHEDPEVKFNWYVDGVEVHNAKTKPREEQYNSTYRVVSVLTVLHQDWLNGKEYKCKVSNKALPAPIEKTISKAKGQPREPQVYTLPPSRDELTKNQVSLTCLVKGFYPSDIAVEWESNGQPENNYKTTPPVLDSDGSFFLYSKLTVDKSRWQQGNVFSCSVMHEALHNHYTQKSLSLSPGK

SEQ ID NO: 110 - protein, 448 aa, synthetic construct
QVQLQQPGAELVRPGTSVKMSCKASGYTFTSYWMHWVKQRPGQGLEWIGDIYPGSDSTNYHEKFKSKATLTVDTSSSTAYMQLSSLTSEDSAVYYCALDSSGYGFAYWGQGTLVTVSAASTKGPSVFPLAPSSKSTSGGTAALGCLVKDYFPEPVTVSWNSGALTSGVHTFPAVLQSSGLYSLSSVVTVPSSSLGTQTYICNVNHKPSNTKVDKKVEPKSCDKTHTCPPCPAPELLGGPSVFLFPPKPKDTLMISRTPEVTCVVVDVSHEDPEVKFNWYVDGVEVHNAKTKPREEQYNSTYRVVSVLTVLHQDWLNGKEYKCKVSNKALPAPIEKTISKAKGQPREPQVYTLPPSRDELTKNQVSLTCLVKGFYPSDIAVEWESNGQPENNYKTTPPVLDSDGSFFLYSKLTVDKSRWQQGNVFSCSVMHEALHNHYTQKSLSLSPGK

SEQ ID NO: 111 - protein, 450 aa, synthetic construct
EVQLVESGGGLVQPGESLKLSCDSNDYEFPSHDMSWVRKTPEKRLELVAAINSDGGNTYYPDTMERRFIISRDNTKRTLYLQMSSLRSEDTALHYCARPRPTIGTTATGSSMSGAQGPRSASTKGPSVFPLAPSSKSTSGGTAALGCLVKDYFPEPVTVSWNSGALTSGVHTFPAVLQSSGLYSLSSVVTVPSSSLGTQTYICNVNHKPSNTKVDKKVEPKSCDKTHTCPPCPAPELLGGPSVFLFPPKPKDTLMISRTPEVTCVVVDVSHEDPEVKFNWYVDGVEVHNAKTKPREEQYNSTYRVVSVLTVLHQDWLNGKEYKCKVSNKALPAPIEKTISKAKGQPREPQVYTLPPSRDELTKNQVSLTCLVKGFYPSDIAVEWESNGQPENNYKTTPPVLDSDGSFFLYSKLTVDKSRWQQGNVFSCSVMHEALHNHYTQKSLSLSPGK

SEQ ID NO: 112 - protein, 214 aa, synthetic construct
SIVMTQSPKFLLVSAGDRVIITCKASQSVSNDVVWYQQKPGQSPKLLIYYGSHRNTGVPTRFTGSGYGTDFTFTISTVQAEDLAVYFCQQDFFSPWTFGGGTKLEIKRTVAAPSVFIFPPSDEQLKSGTASVVCLLNNFYPREAKVQWKVDNALQSGNSQESVTEQDSKDSTYSLSSTLTLSKADYEKHKVYACEVTHQGLSSPVTKSFNRGEC

SEQ ID NO: 113 - protein, 218 aa, synthetic construct
DIVLTQSPASLAVSLGQRATISCRASESVDEYGISFMNWFQQKPGQPPRLLIYSASNQGSGVPARFTGSGSGTDFSLNILPMEEDDTAMYFCQQSKEVPWTFGGGTKLEIKRTVAAPSVFIFPPSDEQLKSGTASVVCLLNNFYPREAKVQWKVDNALQSGNSQESVTEQDSKDSTYSLSSTLTLSKADYEKHKVYACEVTHQGLSSPVTKSFNRGEC

SEQ ID NO: 114 - protein, 214 aa, synthetic construct
SIVMTQTPKFLLVSAGDRVTITCKASQSVSNDVVWYRQKPGQSPKLLIYYASNRYIGVPDRFTGSGYGTDFTFTISTVQAEDLAVYFCQQDYYSPWTFGGGTKLEIKRTVAAPSVFIFPPSDEQLKSGTASVVCLLNNFYPREAKVQWKVDNALQSGNSQESVTEQDSKDSTYSLSSTLTLSKADYEKHKVYACEVTHQGLSSPVTKSFNRGEC

SEQ ID NO: 115 - protein, 219 aa, synthetic construct
DVVMTQSPLSLPVSLGDQASISCRSSQSLVHSNGNTYLHWYLQKPGQSPKLLIYKVSNRFSGVPDRFSGSGSGTDFTLKISRVEAEDLGVYFCSQSTHVPPDVRWRHQAGNQRTVAAPSVFIFPPSDEQLKSGTASVVCLLNNFYPREAKVQWKVDNALQSGNSQESVTEQDSKDSTYSLSSTLTLSKADYEKHKVYACEVTHQGLSSPVTKSFNRGEC

SEQ ID NO: 116 - protein, 214 aa, synthetic construct
DIQMTQTTSSLSASLGDRVTISCRASQDISNSLNWYQQKPDGTVKLLIYYTSRLHSGVPSRFTGSGSGTDYSLTISNLEQEDIATYFCQQGNTLPLTFGAGTKLELKRTVAAPSVFIFPPSDEQLKSGTASVVCLLNNFYPREAKVQWKVDNALQSGNSQESVTEQDSKDSTYSLSSTLTLSKADYEKHKVYACEVTHQGLSSPVTKSFNRGEC

SEQ ID NO: 117 - protein, 214 aa, synthetic construct
DIQMNQSPSSLSASLGDTITITCHANQNIYVWLSWYQQKPGNIPKLLIYEASNLHTGVPSRFSGSGSGTGFTLTISSLQPEDIATYYCQQGQSYPYTFGGGTKLEIKRTVAAPSVFIFPPSDEQLKSGTASVVCLLNNFYPREAKVQWKVDNALQSGNSQESVTEQDSKDSTYSLSSTLTLSKADYEKHKVYACEVTHQGLSSPVTKSFNRGEC

SEQ ID NO: 118 - protein, 220 aa, synthetic construct
DIVMSQSPSSLAVSVGEKVTMSCKSSQSLLYSRNQKNRLAWYQQKPGQSPKLLIYWASTRESGVPDRFTGSGSGTDFTLTISSVKAEDLAVYYCQQYYSYPRTFGGGTNLEIKRTVAAPSVFIFPPSDEQLKSGTASVVCLLNNFYPREAKVQWKVDNALQSGNSQESVTEQDSKDSTYSLSSTLTLSKADYEKHKVYACEVTHQGLSSPVTKSFNRGEC

SEQ ID NO: 119 - protein, 219 aa, synthetic construct
DVLMTQTPLSLPVSLGDQASISCRSSQSIVHTDGNTYLEWYLQKPGQSPKLLIYKVSNRFSGVPDRFSGSGSGTDFTLKISRVEAEDLGVYYCFQGSHVPWTFGGGTKLEIKRTVAAPSVFIFPPSDEQLKSGTASVVCLLNNFYPREAKVQWKVDNALQSGNSQESVTEQDSKDSTYSLSSTLTLSKADYEKHKVYACEVTHQGLSSPVTKSFNRGEC

SEQ ID NO: 120 - protein, 218 aa, synthetic construct
DIVLTQSPASLAVSLGQRATISCRASESVDSYGNSFMHWYQQKPGQPPKLLIYRASNLESGIPARFSGSGSRTDFTLTINPVEADDVATYYCQQSNEDPFTFGSGTKLEIKRTVAAPSVFIFPPSDEQLKSGTASVVCLLNNFYPREAKVQWKVDNALQSGNSQESVTEQDSKDSTYSLSSTLTLSKADYEKHKVYACEVTHQGLSSPVTKSFNRGEC

SEQ ID NO: 121 - protein, 214 aa, synthetic construct
NIVMTQTPKFLLVSAGDRVTITRKASQSVSNDVVWYQQKPGQSPKLLMYYASYRYTGVPDRFTGSGYGTDFTFTISNVQAEDLAVYFCQQDYSSPFTFGSGTKLEIKRTVAAPSVFIFPPSDEQLKSGTASVVCLLNNFYPREAKVQWKVDNALQSGNSQESVTEQDSKDSTYSLSSTLTLSKADYEKHKVYACEVTHQGLSSPVTKSFNRGEC

SEQ ID NO: 122 - protein, 218 aa, synthetic construct
DIVLTQSPASLAVSLGQRATISCRASQSVSTSTYNYMHWYQQKPGQPPKLLIKYASNLESGVPARFSGSGSGTDFTLNIHPVEEEDTATYYCQHSWEIPFTFGSGTKLEIKRTVAAPSVFIFPPSDEQLKSGTASVVCLLNNFYPREAKVQWKVDNALQSGNSQESVTEQDSKDSTYSLSSTLTLSKADYEKHKVYACEVTHQGLSSPVTKSFNRGEC

SEQ ID NO: 123 - protein, 15 aa, synthetic construct
GGGGSGGGGSGGGGS